European Patent Specification EP 3 857 227 B1, published October 25, 2023. Title: METHODS AND COMPOSITIONS FOR REMOVING BIOTIN INTERFERENCE FROM ASSAYS USING CYCLODEXTRIN TRAPS. Applicant: Siemens Healthcare Diagnostics Inc. Application PCT/US2019/051880. The sequence listing filed with the application follows.

SEQUENCE LISTING (2 sequences)

SEQ ID NO: 1 - protein, 128 aa, Gallus gallus
ARKCSLTGKWTNDLGSNMTIGAVNSRGEFTGTYTTAVTATSNEIKESPLHGTENTINKRTQPTFGFTVNWKFSESTTVFTGQCFIDRNGKEVLKTMWLLRSSVNDIGDDWKATRVGINIFTRLRTQKE

SEQ ID NO: 2 - protein, 127 aa, Streptomyces avidinii
AAEAGITGTWYNQLGSTFIVTAGADGALTGTYESAVGNAESRYVLTGRYDSAPATDGSGTALGWTVAWKNNYRNAHSATTWSGQYVGGAEARINTQWLLTSGTTEANAWKSTLVGHDTFTKVKPSAA